European Patent Application EP 4 446 343 A1, published October 16, 2024. Title: 抗体又はその抗原結合性断片. Applicant: 国立大学法人大阪大学. The sequence listing filed with the application follows.

SEQUENCE LISTING (76 sequences)

SEQ ID NO: 1 - protein, 5 aa, synthetic construct
  REGION 1..5: note = 1
EYIIH

SEQ ID NO: 2 - protein, 8 aa, synthetic construct
  REGION 1..8: note = 2
GYTFTEYI

SEQ ID NO: 3 - protein, 17 aa, synthetic construct
  REGION 1..17: note = 3
WFYPGRGIIKYNEKFKD

SEQ ID NO: 4 - protein, 8 aa, synthetic construct
  REGION 1..8: note = 4
FYPGRGII

SEQ ID NO: 5 - protein, 12 aa, synthetic construct
  REGION 1..12: note = 5
HGITTATGAMDY

SEQ ID NO: 6 - protein, 14 aa, synthetic construct
  REGION 1..14: note = 6
ARHGITTATGAMDY

SEQ ID NO: 7 - protein, 16 aa, synthetic construct
  REGION 1..16: note = 7
RSSQSLLHSNGNTYLH

SEQ ID NO: 8 - protein, 11 aa, synthetic construct
  REGION 1..11: note = 8
QSLLHSNGNTY

SEQ ID NO: 9 - protein, 7 aa, synthetic construct
  REGION 1..7: note = 9
KVSNRFS

SEQ ID NO: 10 - skipped

SEQ ID NO: 11 - protein, 9 aa, synthetic construct
  REGION 1..9: note = 11
SQSTHVPFT

SEQ ID NO: 12 - protein, 9 aa, synthetic construct
  REGION 1..9: note = 12
SQSTHVPFT

SEQ ID NO: 13 - protein, 5 aa, synthetic construct
  REGION 1..5: note = 13
SYAMS

SEQ ID NO: 14 - protein, 8 aa, synthetic construct
  REGION 1..8: note = 14
GITFSSYA

SEQ ID NO: 15 - protein, 16 aa, synthetic construct
  REGION 1..16: note = 15
SISSGGSTYYPDSVKG

SEQ ID NO: 16 - protein, 7 aa, synthetic construct
  REGION 1..7: note = 16
ISSGGST

SEQ ID NO: 17 - protein, 9 aa, synthetic construct
  REGION 1..9: note = 17
IWDGSSYGY

SEQ ID NO: 18 - protein, 11 aa, synthetic construct
  REGION 1..11: note = 18
VAIWDGSSYGY

SEQ ID NO: 19 - protein, 16 aa, synthetic construct
  REGION 1..16: note = 19
RSGQSLVHSNGKTYLH

SEQ ID NO: 20 - protein, 11 aa, synthetic construct
  REGION 1..11: note = 20
QSLVHSNGKTY

SEQ ID NO: 21 - protein, 7 aa, synthetic construct
  REGION 1..7: note = 21
KVSNRFS

SEQ ID NO: 22 - skipped

SEQ ID NO: 23 - protein, 9 aa, synthetic construct
  REGION 1..9: note = 23
SQSTHVPFT

SEQ ID NO: 24 - protein, 9 aa, synthetic construct
  REGION 1..9: note = 24
SQSTHVPFT

SEQ ID NO: 25 - protein, 5 aa, synthetic construct
  REGION 1..5: note = 25
SYAMS

SEQ ID NO: 26 - protein, 8 aa, synthetic construct
  REGION 1..8: note = 26
GFIFSSYA

SEQ ID NO: 27 - protein, 16 aa, synthetic construct
  REGION 1..16: note = 27
SIGSGGTTYYPDSVRG

SEQ ID NO: 28 - protein, 7 aa, synthetic construct
  REGION 1..7: note = 28
IGSGGTT

SEQ ID NO: 29 - protein, 9 aa, synthetic construct
  REGION 1..9: note = 29
IWDGSSHGY

SEQ ID NO: 30 - protein, 11 aa, synthetic construct
  REGION 1..11: note = 30
AAIWDGSSHGY

SEQ ID NO: 31 - protein, 16 aa, synthetic construct
  REGION 1..16: note = 31
RSSQNLVHSNGNTYLH

SEQ ID NO: 32 - protein, 11 aa, synthetic construct
  REGION 1..11: note = 32
QNLVHSNGNTY

SEQ ID NO: 33 - protein, 7 aa, synthetic construct
  REGION 1..7: note = 33
KVSNRFS

SEQ ID NO: 34 - skipped

SEQ ID NO: 35 - protein, 9 aa, synthetic construct
  REGION 1..9: note = 35
SQSTHVPYT

SEQ ID NO: 36 - protein, 9 aa, synthetic construct
  REGION 1..9: note = 36
SQSTHVPYT

SEQ ID NO: 37 - protein, 5 aa, synthetic construct
  REGION 1..5: note = 37
SYAMS

SEQ ID NO: 38 - protein, 8 aa, synthetic construct
  REGION 1..8: note = 38
GFTFSSYA

SEQ ID NO: 39 - protein, 17 aa, synthetic construct
  REGION 1..17: note = 39
SINSGGVTTYYPDSVKG

SEQ ID NO: 40 - protein, 8 aa, synthetic construct
  REGION 1..8: note = 40
INSGGVTT

SEQ ID NO: 41 - protein, 9 aa, synthetic construct
  REGION 1..9: note = 41
IWDGSSHGY

SEQ ID NO: 42 - protein, 11 aa, synthetic construct
  REGION 1..11: note = 42
AAIWDGSSHGY

SEQ ID NO: 43 - protein, 16 aa, synthetic construct
  REGION 1..16: note = 43
RSSQSLVHSNGNTYLH

SEQ ID NO: 44 - protein, 11 aa, synthetic construct
  REGION 1..11: note = 44
QSLVHSNGNTY

SEQ ID NO: 45 - protein, 7 aa, synthetic construct
  REGION 1..7: note = 45
KVSNRFS

SEQ ID NO: 46 - skipped

SEQ ID NO: 47 - protein, 9 aa, synthetic construct
  REGION 1..9: note = 47
SQSTHVPYT

SEQ ID NO: 48 - protein, 9 aa, synthetic construct
  REGION 1..9: note = 48
SQSTHVPYT

SEQ ID NO: 49 - protein, 5 aa, synthetic construct
  REGION 1..5: note = 49
DAWMD

SEQ ID NO: 50 - protein, 8 aa, synthetic construct
  REGION 1..8: note = 50
GFTFSDAW

SEQ ID NO: 51 - protein, 19 aa, synthetic construct
  REGION 1..19: note = 51
EIRNKANNHATYFTESVKG

SEQ ID NO: 52 - protein, 10 aa, synthetic construct
  REGION 1..10: note = 52
IRNKANNHAT

SEQ ID NO: 53 - protein, 5 aa, synthetic construct
  REGION 1..5: note = 53
ATFVY

SEQ ID NO: 54 - protein, 7 aa, synthetic construct
  REGION 1..7: note = 54
TTATFVY

SEQ ID NO: 55 - protein, 15 aa, synthetic construct
  REGION 1..15: note = 55
RSSQSLVRNGITYLH

SEQ ID NO: 56 - protein, 10 aa, synthetic construct
  REGION 1..10: note = 56
QSLVRNGITY

SEQ ID NO: 57 - protein, 7 aa, synthetic construct
  REGION 1..7: note = 57
KVSNRFS

SEQ ID NO: 58 - skipped

SEQ ID NO: 59 - protein, 9 aa, synthetic construct
  REGION 1..9: note = 59
SQTPHVPYT

SEQ ID NO: 60 - protein, 9 aa, synthetic construct
  REGION 1..9: note = 60
SQTPHVPYT

SEQ ID NO: 61 - protein, 6 aa, synthetic construct
  REGION 1..6: note = 61
TKVTKF

SEQ ID NO: 62 - protein, 5 aa, synthetic construct
  REGION 1..5: note = 62
EIKRL

SEQ ID NO: 63 - protein, 6 aa, synthetic construct
  REGION 1..6: note = 63
DEEIKR

SEQ ID NO: 64 - protein, 6 aa, synthetic construct
  REGION 1..6: note = 64
IKRLLQ

SEQ ID NO: 65 - protein, 28 aa, Homo sapiens
EVTKVTKFIEGGDGHLFEDEEIKRLLQG

SEQ ID NO: 66 - protein, 809 aa, Homo sapiens
MIPFLPMFSLLLLLIVNPINANNHYDKILAHSRIRGRDQGPNVCALQQILGTKKKYFSTCKNWYKKSICGQKTTVLYECCPGYMRMEGMKGCPAVLPIDHVYGTLGIVGATTTQRYSDASKLREEIEGKGSFTYFAPSNEAWDNLDSDIRRGLESNVNVELLNALHSHMINKRMLTKDLKNGMIIPSMYNNLGLFINHYPNGVVTVNCARIIHGNQIATNGVVHVIDRVLTQIGTSIQDFIEAEDDLSSFRAAAITSDILEALGRDGHFTLFAPTNEAFEKLPRGVLERIMGDKVASEALMKYHILNTLQCSESIMGGAVFETLEGNTIEIGCDGDSITVNGIKMVNKKDIVTNNGVIHLIDQVLIPDSAKQVIELAGKQQTTFTDLVAQLGLASALRPDGEYTLLAPVNNAFSDDTLSMDQRLLKLILQNHILKVKVGLNELYNGQILETIGGKQLRVFVYRTAVCIENSCMEKGSKQGRNGAIHIFREIIKPAEKSLHEKLKQDKRFSTFLSLLEAADLKELLTQPGDWTLFVPTNDAFKGMTSEEKEILIRDKNALQNIILYHLTPGVFIGKGFEPGVTNILKTTQGSKIFLKEVNDTLLVNELKSKESDIMTTNGVIHVVDKLLYPADTPVGNDQLLEILNKLIKYIQIKFVRGSTFKEIPVTVYRPTLTKVKIEGEPEFRLIKEGETITEVIHGEPIIKKYTKIIDGVPVEITEKETREERIITGPEIKYTRISTGGGETEETLKKLLQEEVTKVTKFIEGGDGHLFEDEEIKRLLQGDTPVRKLQANKKVQGSRRRLREGRSQ

SEQ ID NO: 67 - protein, 121 aa, synthetic construct
  REGION 1..121: note = 67
KVQLVQSGAEVVKPGASVKLSCKASGYTFTEYIIHWVKQASGQGLEWIGWFYPGRGIIKYNEKFKDKATLTADKSISTVYMDLSRLRSEDTAVYFCARHGITTATGAMDYWGQGTLVTVSS

SEQ ID NO: 68 - protein, 112 aa, synthetic construct
  REGION 1..112: note = 68
DVVMTQTPLSLSVTLGQPASISCRSSQSLLHSNGNTYLHWYLQKPGQAPKLLIYKVSNRFSGVPDRFSGSGSGTDFTLKISRVEAEDVGVYFCSQSTHVPFTFGQGTKLEIK

SEQ ID NO: 69 - protein, 117 aa, synthetic construct
  REGION 1..117: note = 69
EVQLVESGGGLVKPGGSLRLSCAASGITFSSYAMSWVRQAPGKGLEWVASISSGGSTYYPDSVKGRFTISRDNAKNSLYLQMNSLRAEDTAVYYCVAIWDGSSYGYWGQGTTVTVSS

SEQ ID NO: 70 - protein, 112 aa, synthetic construct
  REGION 1..112: note = 70
DIVMTQTPLSLSVTPGQPASISCKSGQSLVHSNGKTYLHWYLQKPGQSPQLLIYKVSNRFSGVPDRFSGSGSGTDFTLKISRVEAEDVGVYYCSQSTHVPFTFGQGTKLEIK

SEQ ID NO: 71 - protein, 117 aa, synthetic construct
  REGION 1..117: note = 71
EVQLVESGGGLVKPGGSLRLSCAASGFIFSSYAMSWVRQPPGKRLEWVASIGSGGTTYYPDSVRGRFTISRDNARNILYLQMRSLRAEDTAVYYCAAIWDGSSHGYWGQGTLLTVSS

SEQ ID NO: 72 - protein, 112 aa, synthetic construct
  REGION 1..112: note = 72
DVVMTQSPLSLPVTLGQPASISCRSSQNLVHSNGNTYLHWYLQRPGQSPQLLIYKVSNRFSGVPDRFSGSGSGTDFTLKISRVEAEDLGVYYCSQSTHVPYTFGPGTKLEIK

SEQ ID NO: 73 - protein, 118 aa, synthetic construct
  REGION 1..118: note = 73
EVQLVESGGGLVKPGGSLRLSCAASGFTFSSYAMSWVRQTPEKRLEWVASINSGGVTTYYPDSVKGRFTISRDNAINILYLQMRSLRSEDTALYYCAAIWDGSSHGYWGQGTLVTVSS

SEQ ID NO: 74 - protein, 112 aa, synthetic construct
  REGION 1..112: note = 74
DVVMTQSPLSLPVTLGQPASISCRSSQSLVHSNGNTYLHWYLQRPGQSPRLLIYKVSNRFSGVPDRFSGSGSGTDFTLKISRVEAEDFGVYFCSQSTHVPYTFGPGTKLEIK

SEQ ID NO: 75 - protein, 116 aa, synthetic construct
  REGION 1..116: note = 75
EVQLVESGGGLVQPGGSLKLSCAASGFTFSDAWMDWVRQAPGKGLEWVAEIRNKANNHATYFTESVKGRFTISRDDSKNTVYLQMNSLRAEDTAVYYCTTATFVYWGQGTLVTVSS

SEQ ID NO: 76 - protein, 111 aa, synthetic construct
  REGION 1..111: note = 76
DVVMTQSPLSLPVSLGDRASISCRSSQSLVRNGITYLHWYQQKPGQSPKLLIYKVSNRFSGVPDRFSGSGSGTDFTLKISSVEAEDFGVYYCSQTPHVPYTFGQGTKLEIK